European Patent Application EP 4 124 623 A1, published February 1, 2023. Title: CD36 INHIBITOR FOR USE IN PROMOTING MUSCLE REGENERATION. Applicant: Universitat Pompeu Fabra Fundació Institut de Recerca Biomédica Institució Catalana De Recerca I Estudis Avançats. The sequence listing filed with the application follows.

SEQUENCE LISTING (32 sequences)

SEQ ID NO: 1 - RNA, 19 nt, Artificial sequence
  Artificial sequence
ccacauaucuaccaaaauu

SEQ ID NO: 2 - RNA, 19 nt, Artificial sequence
  Artificial sequence
gaaaggauaacauaagcaa

SEQ ID NO: 3 - RNA, 19 nt, Artificial sequence
  Artificial sequence
auacagaguucguuaucua

SEQ ID NO: 4 - RNA, 19 nt, Artificial sequence
  Artificial sequence
ggauuggaguggugauguu

SEQ ID NO: 5 - DNA, 21 bp, Artificial sequence
  Artificial sequence
catctggagcagcatggagtc

SEQ ID NO: 6 - DNA, 22 bp, Artificial sequence
  Artificial sequence
atcatcatcacctgaatcgggg

SEQ ID NO: 7 - DNA, 18 bp, Artificial sequence
  Artificial sequence
gacctcggcgtcgtagtg

SEQ ID NO: 8 - DNA, 20 bp, Artificial sequence
  Artificial sequence
aagggcgagatcaagatgag

SEQ ID NO: 9 - DNA, 23 bp, Artificial sequence
  Artificial sequence
tgaggctagagaggatcttgaga

SEQ ID NO: 10 - DNA, 21 bp, Artificial sequence
  Artificial sequence
gcagaagagctgctacgtgaa

SEQ ID NO: 11 - DNA, 20 bp, Artificial sequence
  Artificial sequence
ccaggccaagatggtgtctt

SEQ ID NO: 12 - DNA, 21 bp, Artificial sequence
  Artificial sequence
tgagaaaggatcagccattgc

SEQ ID NO: 13 - DNA, 21 bp, Artificial sequence
  Artificial sequence
ggtgacaaccacggccttccc

SEQ ID NO: 14 - DNA, 23 bp, Artificial sequence
  Artificial sequence
aagcctccgacttgtgaagtggt

SEQ ID NO: 15 - DNA, 21 bp, Artificial sequence
  Artificial sequence
ccaaaatacctgtggccttgg

SEQ ID NO: 16 - DNA, 20 bp, Artificial sequence
  Artificial sequence
gcttgtgctctgcttgtgag

SEQ ID NO: 17 - DNA, 19 bp, Artificial sequence
  Artificial sequence
ccgatgggctcgagtatga

SEQ ID NO: 18 - DNA, 23 bp, Artificial sequence
  Artificial sequence
ttgtctgatgagttcagcatcca

SEQ ID NO: 19 - DNA, 22 bp, Artificial sequence
  Artificial sequence
cgctcttctgtctactgaactt

SEQ ID NO: 20 - DNA, 18 bp, Artificial sequence
  Artificial sequence
gatgagagggaggccatt

SEQ ID NO: 21 - DNA, 26 bp, Artificial sequence
  Artificial sequence
agcggctgactgaactcagattgtag

SEQ ID NO: 22 - DNA, 24 bp, Artificial sequence
  Artificial sequence
gtcacagttttcagctgtataggg

SEQ ID NO: 23 - DNA, 19 bp, Artificial sequence
  Artificial sequence
tccagcgcaagaaagaaaa

SEQ ID NO: 24 - DNA, 20 bp, Artificial sequence
  Artificial sequence
aatagcgatcctgagcttgc

SEQ ID NO: 25 - DNA, 20 bp, Artificial sequence
  Artificial sequence
cccactcacctgctgctact

SEQ ID NO: 26 - DNA, 20 bp, Artificial sequence
  Artificial sequence
tctggacccattccttcttg

SEQ ID NO: 27 - DNA, 20 bp, Artificial sequence
  Artificial sequence
ctggctgtgaccctctctgt

SEQ ID NO: 28 - DNA, 20 bp, Artificial sequence
  Artificial sequence
atcttccttttggcaagcaa

SEQ ID NO: 29 - DNA, 21 bp, Artificial sequence
  Artificial sequence
gaagctcatctatgagaaggc

SEQ ID NO: 30 - DNA, 21 bp, Artificial sequence
  Artificial sequence
aagacgaaggagctgcagaac

SEQ ID NO: 31 - DNA, 21 bp, Artificial sequence
  Artificial sequence
aacgcaaacgcatgatcactg

SEQ ID NO: 32 - DNA, 20 bp, Artificial sequence
  Artificial sequence
tcagggatgatgcatctagc